European Patent Application EP 4 471 067 A1, published December 4, 2024. Title: A chemically inducible heterodimerizing system and a method for generation thereof. Applicant: Miltenyi Biotec B.V. & Co. KG. Application EP. The sequence listing filed with the application follows.

SEQUENCE LISTING (41 sequences)

SEQ ID NO: 1 - protein, 119 aa, synthetic construct
QVQLVESGGGLVQAGGSLRLSCTASGRTGTIYSMAWFRQAPGKEREFLATVGWSSGITYYMDSVKGRFTISRDKGKNTVYLQMDSLKPEDTAVYYCTATRAYSVGYDYWGQGTQVTVSS

SEQ ID NO: 2 - protein, 119 aa, synthetic construct
QVQLVESGGGLVQAGGSLRLSCTASGRTGTIYSMAWFRQAPGKEREFLATVGWSSGITYYMDSVKGRFTISRDKGKNTVYLQMDSLKPEDTAVYYCTATRAYSDGYDYWGQGTQVTVSS

SEQ ID NO: 3 - protein, 119 aa, synthetic construct
QVQLVESGGGLVQAGGSLRLSCTASGRTGTIYSMAWFRQAPGKEREFLAXXXXXXXXTYYMDSVKGRFTISRDKGKNTVYLQMDSLKPEDTAVYYCTATRAYSVGYDYWGQGTQVTVSS

SEQ ID NO: 4 - protein, 119 aa, synthetic construct
QVQLVESGGGLVQAGGSLRLSCTASGRTGTIYSMAWFRQAPGKEREFLAPVALGLQSTYYMDSVKGRFTISRDKGKNTVYLQMDSLKPEDTAVYYCTATRAYSVGYDYWGQGTQVTVSS

SEQ ID NO: 5 - protein, 119 aa, synthetic construct
QVQLVESGGGLVQAGGSLRLSCTASGRTGTIYSMAWFRQAPGKEREFLAQQRWLFRRTYYMDSVKGRFTISRDKGKNTVYLQMDSLKPEDTAVYYCTATRAYSVGYDYWGQGTQVTVSS

SEQ ID NO: 6 - protein, 119 aa, synthetic construct
QVQLVESGGGLVQAGGSLRLSATAYGKTGTIYSMAWFRQAPGKEREFLAPVALGLQSTYYMDSVKGRFTISRDKGKNTVYLQMDSLKPEDTAVYYAAATRAYSVGYDYWGQGTQVTVTS

SEQ ID NO: 7 - protein, 119 aa, synthetic construct
EVQLVESGGGLVQAGGSLRLSATAYGRTGTIYSMAWFRQAPGKEREFLAPVALGLQSTYYMDSVKGRFTISRDKGKNTVYLQMDSLKPEDTAVYYAAATRAYSVGYDYWGQGTQVTVSS

SEQ ID NO: 8 - protein, 119 aa, synthetic construct
QVQLVESGGGLVQAGGSLRLSCTASGRTGTIYSMAWFRQAPGKEREFLATVGWSSGITYYMDSVKGRFTISRDKGKNTVYLQMDSLKPEDTAVYYCTATRAYSEGYDYWGQGTQVTVSS

SEQ ID NO: 9 - DNA, 42 bp, synthetic construct
  source 1..42: mol_type = other DNA
ggctctggtggaggcggtagcggaggcggagggtcggctagc

SEQ ID NO: 10 - DNA, 42 bp, synthetic construct
  source 1..42: mol_type = other DNA
ctattacaagtcctcttcagaaataagcttttgttcggatcc

SEQ ID NO: 11 - protein, 258 aa, synthetic construct
MQLLRCFSIFSVIASVLAQELTTICEQIPSPTLESTPYSLSTTTILANGKAMQGVFEYYKSVTFVSNCGSHPSTTSKGSPINTQYVFKDNSSTIEGRYPYDVPDYALQASGGGGSGGGGSGGGGSASQVQLVESGGGLVQAGGSLRLSCTASGRTGTIYSMAWFRQAPGKEREFLATVGWSSGITYYMDSVKGRFTISRDKGKNTVYLQMDSLKPEDTAVYYCTATRAYSVGYDYWGQGTQVTVSSGSEQKLISEEDL

SEQ ID NO: 12 - DNA, 24 bp, synthetic construct
  source 1..24: mol_type = other DNA
cgtttgtcagtaattgcggttctc

SEQ ID NO: 13 - DNA, 29 bp, synthetic construct
  source 1..29: mol_type = other DNA
ctgagactgagctggaccgcctctggcag

SEQ ID NO: 14 - DNA, 29 bp, synthetic construct
  source 1..29: mol_type = other DNA
ctgccagaggcggtccagctcagtctcag

SEQ ID NO: 15 - DNA, 32 bp, synthetic construct
  source 1..32: mol_type = other DNA
tctctgagactgagcgctaccgcctctggcag

SEQ ID NO: 16 - DNA, 32 bp, synthetic construct
  source 1..32: mol_type = other DNA
ctgccagaggcggtagcgctcagtctcagaga

SEQ ID NO: 17 - DNA, 36 bp, synthetic construct
  source 1..36: mol_type = other DNA
gatctctgagactgagcgttaccgcctctggcagaa

SEQ ID NO: 18 - DNA, 36 bp, synthetic construct
  source 1..36: mol_type = other DNA
ttctgccagaggcggtaacgctcagtctcagagatc

SEQ ID NO: 19 - DNA, 29 bp, synthetic construct
  source 1..29: mol_type = other DNA
ctctgagactgagcggtaccgcctctggc

SEQ ID NO: 20 - DNA, 29 bp, synthetic construct
  source 1..29: mol_type = other DNA
gccagaggcggtaccgctcagtctcagag

SEQ ID NO: 21 - DNA, 31 bp, synthetic construct
  source 1..31: mol_type = other DNA
ctctgagactgagctttaccgcctctggcag

SEQ ID NO: 22 - DNA, 31 bp, synthetic construct
  source 1..31: mol_type = other DNA
ctgccagaggcggtaaagctcagtctcagag

SEQ ID NO: 23 - DNA, 32 bp, synthetic construct
  source 1..32: mol_type = other DNA
accgccgtgtactacgccacagccacaagagc

SEQ ID NO: 24 - DNA, 32 bp, synthetic construct
  source 1..32: mol_type = other DNA
gctcttgtggctgtggcgtagtacacggcggt

SEQ ID NO: 25 - DNA, 34 bp, synthetic construct
  source 1..34: mol_type = other DNA
caccgccgtgtactacgtcacagccacaagagcc

SEQ ID NO: 26 - DNA, 34 bp, synthetic construct
  source 1..34: mol_type = other DNA
ggctcttgtggctgtgacgtagtacacggcggtg

SEQ ID NO: 27 - DNA, 32 bp, synthetic construct
  source 1..32: mol_type = other DNA
accgccgtgtactaccccacagccacaagagc

SEQ ID NO: 28 - DNA, 32 bp, synthetic construct
  source 1..32: mol_type = other DNA
gctcttgtggctgtggggtagtacacggcggt

SEQ ID NO: 29 - DNA, 29 bp, synthetic construct
  source 1..29: mol_type = other DNA
gccgtgtactactggacagccacaagagc

SEQ ID NO: 30 - DNA, 29 bp, synthetic construct
  source 1..29: mol_type = other DNA
gctcttgtggctgtccagtagtacacggc

SEQ ID NO: 31 - protein, 16 aa, synthetic construct
GSSGGGGSGGGGSSGM

SEQ ID NO: 32 - protein, 10 aa, synthetic construct
SRGSGSGSGS

SEQ ID NO: 33 - protein, 14 aa, synthetic construct
GSGSGSGSGSGSGS

SEQ ID NO: 34 - protein, 515 aa, synthetic construct
MLLLVTSLLLCELPHPAFLLIPDIQMTQTTSSLSASLGDRVTISCRASQDISKYLNWYQQKPDGTVKLLIYHTSRLHSGVPSRFSGSGSGTDYSLTISNLEQEDIATYFCQQGNTLPYTFGGGTKLEITGSTSGSGKPGSGEGSTKGEVKLQESGPGLVAPSQSLSVTCTVSGVSLPDYGVSWIRQPPRKGLEWLGVIWGSETTYYNSALKSRLTIIKDNSKSQVFLKMNSLQTDDTAIYYCAKHYYYGGSYAMDYWGQGTSVTVSSDYKDDDDKTTTPAPRPPTPAPTIASQPLSLRPEACRPAAGGAVHTRGLDFACDIYIWAPLAGTCGVLLLSLVITLYCKRGRKKLLYIFKQPFMRPVQTTQEEDGCSCRFPEEEEGGCELSRGSGSGSGSQVQLVESGGGLVQAGGSLRLSATAYGKTGTIYSMAWFRQAPGKEREFLAPVALGLQSTYYMDSVKGRFTISRDKGKNTVYLQMDSLKPEDTAVYYAAATRAYSVGYDYWGQGTQVTVTS

SEQ ID NO: 35 - protein, 45 aa, synthetic construct
TTTPAPRPPTPAPTIASQPLSLRPEASRPAAGGAVHTRGLDFASD

SEQ ID NO: 36 - protein, 619 aa, synthetic construct
MIHLGHILFLLLLPVAAAQTTPGERSSLPAFYPGTSGSCSGCGSLSLPIYIWAPLAGTCGVLLLSLVITLYCSLKRGRKKLLYIFKQPFMRPVQTTQEEDGCSCRFPEEEEGGCELGSGSGSGSGSGSGSGSQVQLVESGGGLVQAGGSLRLSCTASGRTGTIYSMAWFRQAPGKEREFLATVGWSSGITYYMDSVKGRFTISRDKGKNTVYLQMDSLKPEDTAVYYCTATRAYSDGYDYWGQGTQVTVSSGSGSGSGSSLRVKFSRSADAPAYKQGQNQLYNELNLGRREEYDVLDKRRGRDPEMGGKPRRKNPQEGLYNELQKDKMAEAYSEIGMKGERRRGKGHDGLYQGLSTATKDTYDALHMQALPPRSRGSGSGSGSMVSKGEEDNMAIIKEFMRFKVHMEGSVNGHEFEIEGEGEGRPYEGTQTAKLKVTKGGPLPFAWDILSPQFMYGSKAYVKHPADIPDYLKLSFPEGFKWERVMNFEDGGVVTVTQDSSLQDGEFIYKVKLRGTNFPSDGPVMQKKTMGWEASSERMYPEDGALKGEIKQRLKLKDGGHYDAEVKTTYKAKKPVQLPGAYNVNIKLDITSHNEDYTIVEQYERAEGRHSTGGMDELYK

SEQ ID NO: 37 - protein, 389 aa, synthetic construct
MRTLLTILTVGSLAAHGSNWSHPQFEKTTTPAPRPPTPAPTIASQPLSLRPEASRPAAGGAVHTRGLDFASDIYIWAPLAGTCGVLLLSLVITLYCKRGRKKLLYIFKQPFMRPVQTTQEEDGCSCRFPEEEEGGCELSRGSGSGSGSQVQLVESGGGLVQAGGSLRLSCTASGRTGTIYSMAWFRQAPGKEREFLATVGWSSGITYYMDSVKGRFTISRDKGKNTVYLQMDSLKPEDTAVYYCTATRAYSDGYDYWGQGTQVTVSSGSGSGSGSSLRVKFSRSADAPAYKQGQNQLYNELNLGRREEYDVLDKRRGRDPEMGGKPRRKNPQEGLYNELQKDKMAEAYSEIGMKGERRRGKGHDGLYQGLSTATKDTYDALHMQALPPR

SEQ ID NO: 38 - protein, 504 aa, synthetic construct
MLLLVTSLLLCELPHPAFLLIPDIQMTQTTSSLSASLGDRVTISCRASQDISKYLNWYQQKPDGTVKLLIYHTSRLHSGVPSRFSGSGSGTDYSLTISNLEQEDIATYFCQQGNTLPYTFGGGTKLEITGSTSGSGKPGSGEGSTKGEVKLQESGPGLVAPSQSLSVTCTVSGVSLPDYGVSWIRQPPRKGLEWLGVIWGSETTYYNSALKSRLTIIKDNSKSQVFLKMNSLQTDDTAIYYCAKHYYYGGSYAMDYWGQGTSVTVSSDYKDDDDKTTTPAPRPPTPAPTIASQPLSLRPEACRPAAGGAVHTRGLDFACDIYIWAPLAGTCGVLLLSLVITLYCKRGRKKLLYIFKQPFMRPVQTTQEEDGCSCRFPEEEEGGCELSRGSGSGSGSMGVQVETISPGDGRTFPKRGQTCVVHYTGMLEDGKKFDSSRDRNKPFKFMLGKQEVIRGWEEGVAQMSVGQRAKLTISPDYAYGATGHPGIIPPHATLVFDVELLKLE

SEQ ID NO: 39 - protein, 593 aa, synthetic construct
MIHLGHILFLLLLPVAAAQTTPGERSSLPAFYPGTSGSCSGCGSLSLPIYIWAPLAGTCGVLLLSLVITLYCSLKRGRKKLLYIFKQPFMRPVQTTQEEDGCSCRFPEEEEGGCELGSGSGSGSGSGSGSGSILWHEMWHEGLEEASRLYFGERNVKGMFEVLEPLHAMMERGPQTLKETSFNQAYGRDLMEAQEWCRKYMKSGNVKDLLQAWDLYYHVFRRISKGSGSGSGSSLRVKFSRSADAPAYKQGQNQLYNELNLGRREEYDVLDKRRGRDPEMGGKPRRKNPQEGLYNELQKDKMAEAYSEIGMKGERRRGKGHDGLYQGLSTATKDTYDALHMQALPPRSRGSGSGSGSMVSKGEEDNMAIIKEFMRFKVHMEGSVNGHEFEIEGEGEGRPYEGTQTAKLKVTKGGPLPFAWDILSPQFMYGSKAYVKHPADIPDYLKLSFPEGFKWERVMNFEDGGVVTVTQDSSLQDGEFIYKVKLRGTNFPSDGPVMQKKTMGWEASSERMYPEDGALKGEIKQRLKLKDGGHYDAEVKTTYKAKKPVQLPGAYNVNIKLDITSHNEDYTIVEQYERAEGRHSTGGMDELYK

SEQ ID NO: 40 - protein, 498 aa, synthetic construct
MLLLVTSLLLCELPHPAFLLIPDIQMTQTTSSLSASLGDRVTISCRASQDISKYLNWYQQKPDGTVKLLIYHTSRLHSGVPSRFSGSGSGTDYSLTISNLEQEDIATYFCQQGNTLPYTFGGGTKLEITGSTSGSGKPGSGEGSTKGEVKLQESGPGLVAPSQSLSVTCTVSGVSLPDYGVSWIRQPPRKGLEWLGVIWGSETTYYNSALKSRLTIIKDNSKSQVFLKMNSLQTDDTAIYYCAKHYYYGGSYAMDYWGQGTSVTVSSDYKDDDDKTTTPAPRPPTPAPTIASQPLSLRPEACRPAAGGAVHTRGLDFACDIYIWAPLAGTCGVLLLSLVITLYCKRGRKKLLYIFKQPFMRPVQTTQEEDGCSCRFPEEEEGGCELRVKFSRSADAPAYKQGQNQLYNELNLGRREEYDVLDKRRGRDPEMGGKPRRKNPQEGLYNELQKDKMAEAYSEIGMKGERRRGKGHDGLYQGLSTATKDTYDALHMQALPPR

SEQ ID NO: 41 - protein, 27 aa, synthetic construct
RAKRGSGATNFSLLKQAGDVEENPGPD